European Patent Specification EP 3 813 866 B1, published January 28, 2026. Title: AF for use in treatment and/or prevention of acute respiratory failure. Applicant: Lantmännen AS Faktor AB. The sequence listing filed with the application follows.

SEQUENCE LISTING (6 sequences)

SEQ ID NO: 1 - protein, 382 aa, human
MVLESTMVCVDNSEYMRNGDFLPTRLQAQQDAVNIVCHSKTRSNPENNVGLITLANDCEVLTTLTPDTGRILSKLHTVQPKGKITFCTGIRVAHLALKHRQGKNHKMRIIAFVGSPVEDNEKDLVKLAKRLKKEKVNVDIINFGEEEVNTEKLTAFVNTLNGKDGTGSHLVTVPPGPSLADALISSPILAGEGGAMLGLGASDFEFGVDPSADPELALALRVSMEEQRHAGGGARRAARASAAEAGIATTGTEDSDDALLKMTISQQEFGRTGLPDLSSMTEEEQIAYAMQMSLQGAEFGQAESADIDASSAMDTSEPAKEEDDYDVMQDPEFLQSVLENLPGVDPNNEAIRNAMGSLPPRPPRTARRTRRRKTRSETGGKG

SEQ ID NO: 2 - protein, 6 aa, Artifical sequence
  VARIANT 5: may be replaced by A
  VARIANT 2: may be replaced by R or K
  VARIANT 3: may be replaced by L
  VARIANT 1: may be replaced by S
CHSKTR

SEQ ID NO: 3 - protein, 16 aa, artifical sequence
  VARIANT 6: may be replaced with A
  VARIANT 3: may be replaced with R or K
  VARIANT 4: may be replaced with L
  VARIANT 2: may be replaced by S
VCHSKTRSNPENNVGL

SEQ ID NO: 4 - protein, 7 aa, Artifical sequence
  VARIANT 6: may be replaced by A
  VARIANT 3: may be replaced by R or K
  VARIANT 4: may be replaced by L
  VARIANT 2: may be replaced by S
VCHSKTR

SEQ ID NO: 5 - protein, 8 aa, Artifical Sequence
  VARIANT 7: may be replaced by A
  VARIANT 4: may be replaced by R or K
  VARIANT 5: may be replaced by L
  VARIANT 3: may be replaced by S
IVCHSKTR

SEQ ID NO: 6 - protein, 5 aa, Artifical sequence
  VARIANT 1: may be replaced by R or K
  VARIANT 2: may be replaced by L
  VARIANT 4: may be replaced by A
HSKTR